European Patent Specification EP 3 436 034 B1, published March 26, 2025. Title: MUTANT BORDETELLA STRAINS AND METHODS OF USE. Applicant: INSTITUT PASTEUR DE LILLE INSTITUT NATIONAL DE LA SANTE ET DE LA RECHERCHE MEDICALE (INSERM). The sequence listing filed with the application follows.

SEQUENCE LISTING (8 sequences)

SEQ ID NO: 1 - DNA, 24 bp, Artificial Sequence
  Description of Artificial Sequence: Synthetic primer
atcctcaagcaagactgcgagctg

SEQ ID NO: 2 - DNA, 40 bp, Artificial Sequence
  Description of Artificial Sequence: Synthetic primer
ggggatagaccctcctcgcttggatgccaggtggagagca

SEQ ID NO: 3 - DNA, 40 bp, Artificial Sequence
  Description of Artificial Sequence: Synthetic primer
tgctctccacctggcatccaagcgaggagggtctatcccc

SEQ ID NO: 4 - DNA, 22 bp, Artificial Sequence
  Description of Artificial Sequence: Synthetic primer
ccatcatcctgtacgaccgcct

SEQ ID NO: 5 - DNA, 22 bp, Artificial Sequence
  Description of Artificial Sequence: Synthetic primer
ttcttgcgcgaacagatcaaac

SEQ ID NO: 6 - DNA, 20 bp, Artificial Sequence
  Description of Artificial Sequence: Synthetic primer
ctgctggtcatcggcgaagt

SEQ ID NO: 7 - DNA, 20 bp, Artificial Sequence
  Description of Artificial Sequence: Synthetic primer
cgcccattcttccctgttcc

SEQ ID NO: 8 - DNA, 21 bp, Artificial Sequence
  Description of Artificial Sequence: Synthetic primer
gaacaggaactggaacaggcg